European Patent Application EP 4 538 294 A1, published April 16, 2025. Title: MULTI-SPECIFIC ANTIBODY TARGETING BCMA, GPRC5D AND T CELLS AND APPLICATION THEREOF. Applicant: Shandong Simcere Biopharmaceutical Co.,Ltd. Application US. The sequence listing filed with the application follows.

SEQUENCE LISTING (57 sequences)

SEQ ID NO: 1 - protein, 126 aa, Synthetic construct
EVQLVESGGGLVQPGGSLRLSCSASGFTLDYYMIGWFRQAPGKEREGLSSISPADGSTYYADSVKGRFTISRDSSKNTVYLQMNSLRAEDTAVYYCAAGNEATISWGFGPWEYDYWGQGTMVTVSS

SEQ ID NO: 2 - protein, 123 aa, Synthetic construct
EVQLVESGGGLVQPGGSLRLSCAASESISSIHIMAWYRQAPGKQRELVAGIRNDGSTVYVDSVKGRFTISRDNAKNSLYLQMNSLRAEDTAVYYCNADQGFGSYSEWERRSRWGQGTTVTVSS

SEQ ID NO: 3 - protein, 121 aa, Synthetic construct
EGQMVQSGAEVKKPGSSVKVSCKASGYMFTDHTFHWVRQAPGQGLEWMGYIYPRDQNTKYNEKFKGRVTITADKSTSTAYMELSSLRSEDTAVYYCARAGYYGSSHAMDYWGQGTTVTVSS

SEQ ID NO: 4 - protein, 107 aa, Synthetic construct
DIQMTQSPSSLSASVGDRVTITCKASQDVSTAVAWYQQKPGKSPRLLIYSASSRYTGVPSRFSGSGSGTDFTFTISSLQPEDIATYYCQQLYSTPWTFGGGTKVEIK

SEQ ID NO: 5 - protein, 121 aa, Synthetic construct
EVQLVQSGAEVKKPGSSVKVSCKASGYTFTSYGISWVRQAPGQGLEWMGEIYPRSGNTYYNEKFKGRVTLTADKSTSTAYMELSSLRSEDTAVYYCARGRAYGRNYPMDYWGQGTTVTVSS

SEQ ID NO: 6 - protein, 107 aa, Synthetic construct
EIVLTQSPATLSLSPGERATLSCRASQSIGTSIHWYQQKPGQSPRLLIKYASESISGIPARFSGSGSGTDFTLTISSLEPEDFAVYYCQQSNSWPYTFGGGTKVEIK

SEQ ID NO: 7 - protein, 121 aa, Synthetic construct
EVQLVQSGAEVKKPGASVKVSCKTSGYIFTNFGITWVRQAPGQRLEWMGENYPRRINTYYNEKFKGRVTITADKSASTAYMELSSLRSEDTAVYYCSRKDIFGLSYALDYWGQGTTVTVSS

SEQ ID NO: 8 - protein, 107 aa, Synthetic construct
DIQMTQSPSSLSASVGDRVTITCKASQNVGTNVAWYQHKPGKSPKALIYSASYQYSGVPSRFSGSGSGTDFTLTISSLQPEDVATYICQQYKNYPYTFGGGTKVEIK

SEQ ID NO: 9 - protein, 123 aa, Synthetic construct
EVQLVESGGGVVQPGRSLRLSCAASGFTFTDYYMSWVRQAPGKGLEWVAMSRNKAKGHTIEYSSSVKGRFTISRDNSKNTLYLQMNSLRAEDTAVYYCARDTYESYDGYFDVWGQGTTVTVSS

SEQ ID NO: 10 - protein, 112 aa, Synthetic construct
DIVMTQSPDSLAVSLGERATINCKSSQSLFNSRSRKNYLAWYQQKPGQTPKLLIYWASIRESGVPDRFSGSGSGTDFTLTISSLQAEDVAVYYCKQSYYLYTFGQGTKLEIK

SEQ ID NO: 11 - protein, 231 aa, Synthetic construct
EPKSSDKTHTCPPCPAPEAAGGPSVFLFPPKPKDTLMISRTPEVTCVVVDVSHEDPEVKFNWYVDGVEVHNAKTKPREEQYNSTYRVVSVLTVLHQDWLNGKEYKCKVSNKALPAPIEKTISKAKGQPREPQVYTLPPSREEMTKNQVSLWCLVKGFYPSDIAVEWESNGQPENNYKTTPPVLDSDGSFFLYSKLTVDKSRWQQGNVFSCSVMHEALHNHYTQKSLSLSPG

SEQ ID NO: 12 - protein, 231 aa, Synthetic construct
EPKSSDKTHTCPPCPAPEAAGGPSVFLFPPKPKDTLMISRTPEVTCVVVDVSHEDPEVKFNWYVDGVEVHNAKTKPREEQYNSTYRVVSVLTVLHQDWLNGKEYKCKVSNKALPAPIEKTISKAKGQPREPQVYTLPPSREEMTKNQVSLSCAVKGFYPSDIAVEWESNGQPENNYKTTPPVLDSDGSFFLVSKLTVDKSRWQQGNVFSCSVMHEALHNHYTQKSLSLSPG

SEQ ID NO: 13 - protein, 229 aa, Synthetic construct
ESKYGPPCPPCPAPEAAGGPSVFLFPPKPKDTLMISRTPEVTCVVVDVSQEDPEVQFNWYVDGVEVHNAKTKPREEQFNSTYRVVSVLTVLHQDWLNGKEYKCKVSNKGLPSSIEKTISKAKGQPREPQVYTLPPSQEEMTKNQVSLTCLVKGFYPSDIAVEWESNGQPENNYKTTPPVLDSDGSFFLYSRLTVDKSRWQEGNVFSCSVMHEALHNHYTQKSLSLSLGK

SEQ ID NO: 14 - protein, 228 aa, Synthetic construct
ESKYGPPCPPCPAPEAAGGPSVFLFPPKPKDTLMISRTPEVTCVVVDVSQEDPEVQFNWYVDGVEVHNAKTKPREEQFNSTYRVVSVLTVLHQDWLNGKEYKCKVSNKGLPSSIEKTISKAKGQPREPQVYTLPPSQEEMTKNQVSLWCLVKGFYPSDIAVEWESNGQPENNYKTTPPVLDSDGSFFLYSRLTVDKSRWQEGNVFSCSVMHEALHNHYTQKSLSLSLG

SEQ ID NO: 15 - protein, 228 aa, Synthetic construct
ESKYGPPCPPCPAPEAAGGPSVFLFPPKPKDTLMISRTPEVTCVVVDVSQEDPEVQFNWYVDGVEVHNAKTKPREEQFNSTYRVVSVLTVLHQDWLNGKEYKCKVSNKGLPSSIEKTISKAKGQPREPQVYTLPPSQEEMTKNQVSLSCAVKGFYPSDIAVEWESNGQPENNYKTTPPVLDSDGSFFLVSRLTVDKSRWQEGNVFSCSVMHEALHNHYTQKSLSLSLG

SEQ ID NO: 16 - protein, 98 aa, Synthetic construct
ASTKGPSVFPLAPSSKSTSGGTAALGCLVKDYFPEPVTVSWNSGALTSGVHTFPAVLQSSGLYSLSSVVTVPSSSLGTQTYICNVNHKPSNTKVDKKV

SEQ ID NO: 17 - protein, 98 aa, Synthetic construct
ASTKGPSVFPLAPCSRSTSESTAALGCLVKDYFPEPVTVSWNSGALTSGVHTFPAVLQSSGLYSLSSVVTVPSSSLGTKTYTCNVDHKPSNTKVDKRV

SEQ ID NO: 18 - protein, 451 aa, Synthetic construct
EVQLVESGGGLVQPGGSLRLSCAASGFTFSNFWMTWVRQAPGKGLEWVANMNQDGSEKYYVDSVKGRFTISRDNAKSSLYLQMNSLRAEDTAVYYCARDREYCISTSCYDDFDYWGQGTLVTVSSASTKGPSVFPLAPCSRSTSESTAALGCLVKDYFPEPVTVSWNSGALTSGVHTFPAVLQSSGLYSLSSVVTVPSSSLGTKTYTCNVDHKPSNTKVDKRVESKYGPPCPPCPAPPVAGPSVFLFPPKPKDTLMISRTPEVTCVVVDVSQEDPEVQFNWYVDGVEVHNAKTKPREEQFNSTYRVVSVLTVLHQDWLNGKEYKCKVSNKGLPSSIEKTISKAKGQPREPQVYTLPPSQEEMTKNQVSLTCLVKGFYPSDIAVEWESNGQPENNYKTTPPVLDSDGSFFLYSRLTVDKSRWQEGNVFSCSVMHEALHNHYTQKSLSLSLGK

SEQ ID NO: 19 - protein, 450 aa, Synthetic construct
EVQLVESGGGLVQPGRSLRLSCAASGFTFDDYSMHWVRQAPGKGLEWVSGISWNSGSIGYADSVKGRFTISRDNAKNSLYLQMNSLRAEDTALYYCAKYGSGYGKFYYYGMDVWGQGTTVTVSSASTKGPSVFPLAPCSRSTSESTAALGCLVKDYFPEPVTVSWNSGALTSGVHTFPAVLQSSGLYSLSSVVTVPSSSLGTKTYTCNVDHKPSNTKVDKRVESKYGPPCPPCPAPPVAGPSVFLFPPKPKDTLMISRTPEVTCVVVDVSQEDPEVQFNWYVDGVEVHNAKTKPREEQFNSTYRVVSVLTVLHQDWLNGKEYKCKVSNKGLPSSIEKTISKAKGQPREPQVYTLPPSQEEMTKNQVSLTCLVKGFYPSDIAVEWESNGQPENNYKTTPPVLDSDGSFFLYSRLTVDKSRWQEGNVFSCSVMHEALHNRFTQKSLSLSLGK

SEQ ID NO: 20 - protein, 215 aa, Synthetic construct
DIQMTQSPSSLSASVGDRVTITCRASQSISSYLNWYQQKPGKAPKLLIYAASSLQSGVPSRFSGSGSGTDFTLTISSLQPEDFATYYCQQSYSTPPITFGQGTRLEIKRTVAAPSVFIFPPSDEQLKSGTASVVCLLNNFYPREAKVQWKVDNALQSGNSQESVTEQDSKDSTYSLSSTLTLSKADYEKHKVYACEVTHQGLSSPVTKSFNRGEC

SEQ ID NO: 21 - protein, 445 aa, Synthetic construct
QVQLVQSGAEVKKPGASVKVSCKASGYSFTGYTMNWVRQAPGQGLEWMGLINPYNSDTNYAQKLQGRVTMTTDTSTSTAYMELRSLRSDDTAVYYCARVALRVALDYWGQGTLVTVSSASTKGPSVFPLAPCSRSTSESTAALGCLVKDYFPEPVTVSWNSGALTSGVHTFPAVLQSSGLYSLSSVVTVPSSSLGTKTYTCNVDHKPSNTKVDKRVESKYGPPCPPCPAPEAAGGPSVFLFPPKPKDTLMISRTPEVTCVVVDVSQEDPEVQFNWYVDGVEVHNAKTKPREEQFNSTYRVVSVLTVLHQDWLNGKEYKCKVSNKGLPSSIEKTISKAKGQPREPQVYTLPPSQEEMTKNQVSLTCLVKGFYPSDIAVEWESNGQPENNYKTTPPVLDSDGSFFLYSRLTVDKSRWQEGNVFSCSVMHEALHNHYTQKSLSLSLGK

SEQ ID NO: 22 - protein, 214 aa, Synthetic construct
DIQMTQSPSSLSASVGDRVTITCKASQNVATHVGWYQQKPGKAPKRLIYSASYRYSGVPSRFSGSGSGTEFTLTISNLQPEDFATYYCQQYNRYPYTFGQGTKLEIKRTVAAPSVFIFPPSDEQLKSGTASVVCLLNNFYPREAKVQWKVDNALQSGNSQESVTEQDSKDSTYSLSSTLTLSKADYEKHKVYACEVTHQGLSSPVTKSFNRGEC

SEQ ID NO: 23 - protein, 452 aa, Synthetic construct
EVQLVESGGGLVQPGGSLRLSCAASGFTFNTYAMNWVRQAPGKGLEWVARIRSKYNNYATYYAASVKGRFTISRDDSKNSLYLQMNSLKTEDTAVYYCARHGNFGNSYVSWFAYWGQGTLVTVSSASTKGPSVFPLAPCSRSTSESTAALGCLVKDYFPEPVTVSWNSGALTSGVHTFPAVLQSSGLYSLSSVVTVPSSSLGTKTYTCNVDHKPSNTKVDKRVESKYGPPCPPCPAPEAAGGPSVFLFPPKPKDTLMISRTPEVTCVVVDVSQEDPEVQFNWYVDGVEVHNAKTKPREEQFNSTYRVVSVLTVLHQDWLNGKEYKCKVSNKGLPSSIEKTISKAKGQPREPQVYTLPPSQEEMTKNQVSLTCLVKGFYPSDIAVEWESNGQPENNYKTTPPVLDSDGSFLLYSKLTVDKSRWQEGNVFSCSVMHEALHNHYTQKSLSLSLGK

SEQ ID NO: 24 - protein, 215 aa, Synthetic construct
QTVVTQEPSLTVSPGGTVTLTCRSSTGAVTTSNYANWVQQKPGQAPRGLIGGTNKRAPGTPARFSGSLLGGKAALTLSGVQPEDEAEYYCALWYSNLWVFGGGTKLTVLGQPKAAPSVTLFPPSSEELQANKATLVCLISDFYPGAVTVAWKADSSPVKAGVETTTPSKQSNNKYAASSYLSLTPEQWKSHRSYSCQVTHEGSTVEKTVAPTECS

SEQ ID NO: 25 - protein, 710 aa, Synthetic construct
EVKLDETGGGLVQPGRPMKLSCVASGFTFSDYWMNWVRQSPEKGLEWVAQIRNKPYNYETYYSDSVKGRFTISRDDSKSSVYLQMNNLRVEDMGIYYCTGSYYGMDYWGQGTSVTVSSASTKGPSVFPLAPCSRSTSESTAALGCLVKDYFPEPVTVSWNSGALTSGVHTFPAVLQSSGLYSLSSVVTVPSSSLGTKTYTCNVDHKPSNTKVDKRVGGGGSGGGGSGGGGSEVQLVESGGGVVQPGRSLRLSCAASGFTFTDYYMSWVRQAPGKGLEWVAMSRNKAKGHTIEYSSSVKGRFTISRDNSKNTLYLQMNSLRAEDTAVYYCARDTYESYDGYFDVWGQGTTVTVSSGGGGSGGGGSGGGGSDIVMTQSPDSLAVSLGERATINCKSSQSLFNSRSRKNYLAWYQQKPGQTPKLLIYWASIRESGVPDRFSGSGSGTDFTLTISSLQAEDVAVYYCKQSYYLYTFGQGTKLEIKESKYGPPCPPCPAPEAAGGPSVFLFPPKPKDTLMISRTPEVTCVVVDVSQEDPEVQFNWYVDGVEVHNAKTKPREEQFNSTYRVVSVLTVLHQDWLNGKEYKCKVSNKGLPSSIEKTISKAKGQPREPQVYTLPPSQEEMTKNQVSLTCLVKGFYPSDIAVEWESNGQPENNYKTTPPVLDSDGSFFLYSRLTVDKSRWQEGNVFSCSVMHEALHNHYTQKSLSLSLGK

SEQ ID NO: 26 - protein, 219 aa, Synthetic construct
DVVMTQTPLSLPVSLGDQASISCRSSQSLVHSNGNTYLRWYLQKPGQSPKVLIYKVSNRFSGVPDRFSGSGSGTDFTLKISRVEAEDLGVYFCSQSTHVPWTFGGGTKLEIKRTVAAPSVFIFPPSDEQLKSGTASVVCLLNNFYPREAKVQWKVDNALQSGNSQESVTEQDSKDSTYSLSSTLTLSKADYEKHKVYACEVTHQGLSSPVTKSFNRGEC

SEQ ID NO: 27 - protein, 5 aa, Synthetic construct
YYMIG

SEQ ID NO: 28 - protein, 17 aa, Synthetic construct
SISPADGSTYYADSVKG

SEQ ID NO: 29 - protein, 17 aa, Synthetic construct
GNEATISWGFGPWEYDY

SEQ ID NO: 30 - protein, 5 aa, Synthetic construct
IHIMA

SEQ ID NO: 31 - protein, 16 aa, Synthetic construct
GIRNDGSTVYVDSVKG

SEQ ID NO: 32 - protein, 15 aa, Synthetic construct
DQGFGSYSEWERRSR

SEQ ID NO: 33 - protein, 5 aa, Synthetic construct
DHTFH

SEQ ID NO: 34 - protein, 17 aa, Synthetic construct
YIYPRDQNTKYNEKFKG

SEQ ID NO: 35 - protein, 12 aa, Synthetic construct
AGYYGSSHAMDY

SEQ ID NO: 36 - protein, 11 aa, Synthetic construct
KASQDVSTAVA

SEQ ID NO: 37 - protein, 7 aa, Synthetic construct
SASSRYT

SEQ ID NO: 38 - protein, 9 aa, Synthetic construct
QQLYSTPWT

SEQ ID NO: 39 - protein, 5 aa, Synthetic construct
SYGIS

SEQ ID NO: 40 - protein, 17 aa, Synthetic construct
EIYPRSGNTYYNEKFKG

SEQ ID NO: 41 - protein, 12 aa, Synthetic construct
GRAYGRNYPMDY

SEQ ID NO: 42 - protein, 11 aa, Synthetic construct
RASQSIGTSIH

SEQ ID NO: 43 - protein, 7 aa, Synthetic construct
YASESIS

SEQ ID NO: 44 - protein, 9 aa, Synthetic construct
QQSNSWPYT

SEQ ID NO: 45 - protein, 5 aa, Synthetic construct
NFGIT

SEQ ID NO: 46 - protein, 17 aa, Synthetic construct
ENYPRRINTYYNEKFKG

SEQ ID NO: 47 - protein, 12 aa, Synthetic construct
KDIFGLSYALDY

SEQ ID NO: 48 - protein, 11 aa, Synthetic construct
KASQNVGTNVA

SEQ ID NO: 49 - protein, 7 aa, Synthetic construct
SASYQYS

SEQ ID NO: 50 - protein, 9 aa, Synthetic construct
QQYKNYPYT

SEQ ID NO: 51 - protein, 5 aa, Synthetic construct
DYYMS

SEQ ID NO: 52 - protein, 19 aa, Synthetic construct
MSRNKAKGHTIEYSSSVKG

SEQ ID NO: 53 - protein, 12 aa, Synthetic construct
DTYESYDGYFDV

SEQ ID NO: 54 - protein, 17 aa, Synthetic construct
KSSQSLFNSRSRKNYLA

SEQ ID NO: 55 - protein, 7 aa, Synthetic construct
WASIRES

SEQ ID NO: 56 - protein, 8 aa, Synthetic construct
KQSYYLYT

SEQ ID NO: 57 - protein, 19 aa, Synthetic construct
MGWSWILLFLLSVTAGVHS